European Patent Application EP 4 566 631 A1, published June 11, 2025. Title: New Antibody drug conjugate as well as methods of production and uses thereof. Applicant: Heidelberg Pharma Research GmbH. Application EP, filed December 6, 2023. The sequence listing filed with the application follows.

SEQUENCE LISTING (44 sequences)

SEQ ID NO: 1 - protein, 11 aa, synthetic construct
RASQSISSYLN

SEQ ID NO: 2 - protein, 7 aa, synthetic construct
AASSLQS

SEQ ID NO: 3 - protein, 9 aa, synthetic construct
QQSYSTPWT

SEQ ID NO: 4 - protein, 5 aa, synthetic construct
SSAMH

SEQ ID NO: 5 - protein, 17 aa, synthetic construct
LINPGNGNTKYSQKFQG

SEQ ID NO: 6 - protein, 10 aa, synthetic construct
AYFRGLGFDI

SEQ ID NO: 7 - protein, 9 aa, synthetic construct
QQSYSTPLT

SEQ ID NO: 8 - protein, 14 aa, synthetic construct
TGTSSDVGSYNLVS

SEQ ID NO: 9 - protein, 7 aa, synthetic construct
EGSKRPS

SEQ ID NO: 10 - protein, 9 aa, synthetic construct
SYVPRSSLV

SEQ ID NO: 11 - protein, 5 aa, synthetic construct
TYTIN

SEQ ID NO: 12 - protein, 17 aa, synthetic construct
RIIPVLGIANYAQKFQG

SEQ ID NO: 13 - protein, 13 aa, synthetic construct
DTPRLRSSYYMDV

SEQ ID NO: 14 - protein, 23 aa, synthetic construct
DIQMTQSPSSLSASAGDRVTITC

SEQ ID NO: 15 - protein, 15 aa, synthetic construct
WYQQKPGKAPKLLIY

SEQ ID NO: 16 - protein, 32 aa, synthetic construct
GVPSRFSGSGSGTDFTLAISSLQPEDFATYYC

SEQ ID NO: 17 - protein, 10 aa, synthetic construct
FGQGTKVDIK

SEQ ID NO: 18 - protein, 30 aa, synthetic construct
QVQLVQSGAEVKKPGASVKVSCKASGYIFI

SEQ ID NO: 19 - protein, 14 aa, synthetic construct
WVRQAPGQRLEWMG

SEQ ID NO: 20 - protein, 32 aa, synthetic construct
RVTITRDTSASTAYMELSSLRSEDTAVYYCAR

SEQ ID NO: 21 - protein, 11 aa, synthetic construct
WGQGTLVTVSS

SEQ ID NO: 22 - protein, 23 aa, synthetic construct
DIRMTQSPSSLSASAGDRVTITC

SEQ ID NO: 23 - protein, 32 aa, synthetic construct
GVPSRFSGSGSGTDFTLTISSLQPEDFATYYC

SEQ ID NO: 24 - protein, 10 aa, synthetic construct
FGGGTKLEIK

SEQ ID NO: 25 - protein, 22 aa, synthetic construct
QSALTQPASVSGSPGQSITISC

SEQ ID NO: 26 - protein, 15 aa, synthetic construct
WYQQHPGKAPKLMIY

SEQ ID NO: 27 - protein, 32 aa, synthetic construct
GVSNRFSASKSGNTASLTISGLQTEDEADYYC

SEQ ID NO: 28 - protein, 10 aa, synthetic construct
FGGGTKLTVL

SEQ ID NO: 29 - protein, 30 aa, synthetic construct
QVQLVQSGAEVKKPGSSVKVSCKASGGTFS

SEQ ID NO: 30 - protein, 14 aa, synthetic construct
WVRQAPGQGLEWMG

SEQ ID NO: 31 - protein, 32 aa, synthetic construct
RVTITADKSTSTAYMELSSLRSEDTAVYYCAR

SEQ ID NO: 32 - protein, 107 aa, synthetic construct
DIQMTQSPSSLSASAGDRVTITCRASQSISSYLNWYQQKPGKAPKLLIYAASSLQSGVPSRFSGSGSGTDFTLAISSLQPEDFATYYCQQSYSTPWTFGQGTKVDIK

SEQ ID NO: 33 - protein, 119 aa, synthetic construct
QVQLVQSGAEVKKPGASVKVSCKASGYIFISSAMHWVRQAPGQRLEWMGLINPGNGNTKYSQKFQGRVTITRDTSASTAYMELSSLRSEDTAVYYCARAYFRGLGFDIWGQGTLVTVSS

SEQ ID NO: 34 - protein, 107 aa, synthetic construct
DIRMTQSPSSLSASAGDRVTITCRASQSISSYLNWYQQKPGKAPKLLIYAASSLQSGVPSRFSGSGSGTDFTLTISSLQPEDFATYYCQQSYSTPLTFGGGTKLEIK

SEQ ID NO: 35 - protein, 119 aa, synthetic construct; identical to SEQ ID NO: 33

SEQ ID NO: 36 - protein, 110 aa, synthetic construct
QSALTQPASVSGSPGQSITISCTGTSSDVGSYNLVSWYQQHPGKAPKLMIYEGSKRPSGVSNRFSASKSGNTASLTISGLQTEDEADYYCSSYVPRSSLVFGGGTKLTVL

SEQ ID NO: 37 - protein, 122 aa, synthetic construct
QVQLVQSGAEVKKPGSSVKVSCKASGGTFSTYTINWVRQAPGQGLEWMGRIIPVLGIANYAQKFQGRVTITADKSTSTAYMELSSLRSEDTAVYYCARDTPRLRSSYYMDVWGQGTLVTVSS

SEQ ID NO: 38 - protein, 330 aa, synthetic construct [sequence omitted]

SEQ ID NO: 39 - protein, 449 aa, synthetic construct
QVQLVQSGAEVKKPGASVKVSCKASGYIFISSAMHWVRQAPGQRLEWMGLINPGNGNTKYSQKFQGRVTITRDTSASTAYMELSSLRSEDTAVYYCARAYFRGLGFDIWGQGTLVTVSSASTKGPSVFPLAPSSKSTSGGTAALGCLVKDYFPEPVTVSWNSGALTSGVHTFPAVLQSSGLYSLSSVVTVPSSSLGTQTYICNVNHKPSNTKVDKKVEPKSCDKTHTCPPCPAPELLGGPSVFLFPPKPKDTLMISRTPEVTCVVVCVSHEDPEVKFNWYVDGVEVHNAKTKPREEQYNSTYRVVSVLTVLHQDWLNGKEYKCKVSNKALPAPIEKTISKAKGQPREPQVYTLPPSREEMTKNQVSLTCLVKGFYPSDIAVEWESNGQPENNYKTTPPVLDSDGSFFLYSKLTVDKSRWQQGNVFSCSVMHEALHNHYTQKSLSLSPGK

SEQ ID NO: 40 - protein, 449 aa, synthetic construct; identical to SEQ ID NO: 39

SEQ ID NO: 41 - protein, 452 aa, synthetic construct
QVQLVQSGAEVKKPGSSVKVSCKASGGTFSTYTINWVRQAPGQGLEWMGRIIPVLGIANYAQKFQGRVTITADKSTSTAYMELSSLRSEDTAVYYCARDTPRLRSSYYMDVWGQGTLVTVSSASTKGPSVFPLAPSSKSTSGGTAALGCLVKDYFPEPVTVSWNSGALTSGVHTFPAVLQSSGLYSLSSVVTVPSSSLGTQTYICNVNHKPSNTKVDKKVEPKSCDKTHTCPPCPAPELLGGPSVFLFPPKPKDTLMISRTPEVTCVVVCVSHEDPEVKFNWYVDGVEVHNAKTKPREEQYNSTYRVVSVLTVLHQDWLNGKEYKCKVSNKALPAPIEKTISKAKGQPREPQVYTLPPSREEMTKNQVSLTCLVKGFYPSDIAVEWESNGQPENNYKTTPPVLDSDGSFFLYSKLTVDKSRWQQGNVFSCSVMHEALHNHYTQKSLSLSPGK

SEQ ID NO: 42 - protein, 449 aa, synthetic construct
QVQLVQSGAEVKKPGASVKVSCKASGYIFISSAMHWVRQAPGQRLEWMGLINPGNGNTKYSQKFQGRVTITRDTSASTAYMELSSLRSEDTAVYYCARAYFRGLGFDIWGQGTLVTVSSASTKGPSVFPLAPSSKSTSGGTAALGCLVKDYFPEPVTVSWNSGALTSGVHTFPAVLQSSGLYSLSSVVTVPSSSLGTQTYICNVNHKPSNTKVDKKVEPKSCDKTHTCPPCPAPEAAGGPSVFLFPPKPKDTLMISRTPEVTCVVVCVSHEDPEVKFNWYVDGVEVHNAKTKPREEQYNSTYRVVSVLTVLHQDWLNGKEYKCKVSNKALPAPIEKTISKAKGQPREPQVYTLPPSREEMTKNQVSLTCLVKGFYPSDIAVEWESNGQPENNYKTTPPVLDSDGSFFLYSKLTVDKSRWQQGNVFSCSVMHEALHNHYTQKSLSLSPGK

SEQ ID NO: 43 - protein, 449 aa, synthetic construct; identical to SEQ ID NO: 42

SEQ ID NO: 44 - protein, 461 aa, synthetic construct
QVQLVQSGAEVKKPGSSVKVSCKASGGTFSTYTINWVRQAPGQGLEWMGRIIPVLGIANYAQKFQGRVTITADKSTSTAYMELSSLRSEDTAVYYCARDTPRLRSSYYMDVWGQGTLVTVSSASTKGPSVFPLAPSSKSTSGGTAALGCLVKDYFPEPVTVSWNSGALTSGVHTFPAVLQSSGLYSLSSVVTVPSSSLGTQTYICNVNHKPSNTKVDKKVEPKSCDKTHTCPPCPAPEAAGGPSVFLFPPKPKDTLMISRTPEVTCVVVCVSHEDPEVKFNWYVDGVEVHNAKTKPREEQYNSTYRVVSVLTVLHQDWLNGKEYKCKVSNKALPAPIEKTISKAKGQPREPQVYTLPPSREEMTKNQVSLTCLVKGFYPSDIAVEWESNGQPENNYKTTPPVLDSDGSFFLYSKLTVDKSRWQQGNVFSCSVMHEALHNHYTQKSLSLSPGKMABLALADC